European Patent Specification EP 3 453 768 B1, published March 26, 2025. Title: A METHOD FOR DETECTING TARGET NUCLEIC ACID SEQUENCE USING CLEAVED COMPLEMENTARY TAG FRAGMENT AND A COMPOSITION THEREFOR. Applicant: GeneMatrix Inc. The sequence listing filed with the application follows.

SEQUENCE LISTING (232 sequences)

SEQ ID NO: 1 - DNA, 47 bp, Artificial Sequence
  primer
tgaactatcctggtccgacgtttcggttgtgttgaaacaccgcccgg

SEQ ID NO: 2 - DNA, 22 bp, Artificial Sequence
  primer
gctccttattcggtttgaccgg

SEQ ID NO: 3 - DNA, 41 bp, Artificial Sequence
  primer
atctatgatacctggtttagctcctattgccaacgtattgg

SEQ ID NO: 4 - DNA, 28 bp, Artificial Sequence
  primer
tgtgtggagcatcttgtaatctttggtc

SEQ ID NO: 5 - DNA, 117 bp, Artificial Sequence
  product
tgaactatcctggtccgacgtttcggttgtgttgaaacaccgcccggaacccgatataatccgcccttcaacatcagtgaaaatcttttttttaaccggtcaaaccgaataaggagc

SEQ ID NO: 6 - DNA, 125 bp, Artificial Sequence
  product
atctatgatacctggtttagctcctattgccaacgtattggaaaaaaactttggtattgaaaaaggatttatgacaacagtccactcatatacagcagaccaaagattacaagatgctccacaca

SEQ ID NO: 7 - DNA, 13 bp, Artificial Sequence
  CCTF
ccaggatagttca

SEQ ID NO: 8 - DNA, 15 bp, Artificial Sequence
  CCTF
ccaggtatcatagat

SEQ ID NO: 9 - DNA, 47 bp, Artificial Sequence
  primer
ccactccagccggctgacaccaggacttggtgtgacgctatcagcat

SEQ ID NO: 10 - DNA, 29 bp, Artificial Sequence
  primer
gttttcaaaacacggtcgaaaacaaagtc

SEQ ID NO: 11 - DNA, 46 bp, Artificial Sequence
  primer
catcgccacgagccggttaaccaggttgaaacaccgcccggaaccc

SEQ ID NO: 12 - DNA, 23 bp, Artificial Sequence
  primer
gctccttattcggtttgaccggt

SEQ ID NO: 13 - DNA, 51 bp, Artificial Sequence
  primer
actcacgctaatggagcgcaccaggtttagctcctattgccaacgtattgg

SEQ ID NO: 14 - DNA, 28 bp, Artificial Sequence
  primer
tgtgtggagcatcttgtaatctttggtc

SEQ ID NO: 15 - DNA, 52 bp, Artificial Sequence
  primer
gctacccagccggctacaagccaggctttatggtgcttatattggtggcatg

SEQ ID NO: 16 - DNA, 24 bp, Artificial Sequence
  primer
ctgtataacgttgtgcagcaggtc

SEQ ID NO: 17 - DNA, 47 bp, Artificial Sequence
  primer
tgccgcgtgattcgatcccaccaggtatgtccggcacaacatgcgct

SEQ ID NO: 18 - DNA, 23 bp, Artificial Sequence
  primer
gagcttacgaaggtcggagttga

SEQ ID NO: 19 - DNA, 51 bp, Artificial Sequence
  primer
tctcatagctgggccgctgccaggaagtagcatatgatgaagcacacaaca

SEQ ID NO: 20 - DNA, 25 bp, Artificial Sequence
  primer
taatgcaacgtgcatttgcttcaac

SEQ ID NO: 21 - DNA, 55 bp, Artificial Sequence
  primer
cagatcgttggcactctgcgaccaggttaaagtagcatatgatcaagctcattca

SEQ ID NO: 22 - DNA, 31 bp, Artificial Sequence
  primer
ttgtaatgatacaacgagcatcatcattaat

SEQ ID NO: 23 - DNA, 51 bp, Artificial Sequence
  primer
gctcgtatgccgctccatataccaggccaaatctggatcttcctctgcatc

SEQ ID NO: 24 - DNA, 21 bp, Artificial Sequence
  primer
gagcttgagctggacccagag

SEQ ID NO: 25 - DNA, 48 bp, Artificial Sequence
  primer
acgtgccgtgcatcgttgcaccaggcaaccggctccattttggtggag

SEQ ID NO: 26 - DNA, 21 bp, Artificial Sequence
  primer
cgtcacgtccttcatcggtcc

SEQ ID NO: 27 - DNA, 46 bp, Artificial Sequence
  primer
tcgcagtcccgtcgaggaaccaggaggcctggctatccggagaaac

SEQ ID NO: 28 - DNA, 20 bp, Artificial Sequence
  primer
cgttgtgttggccgcaggtc

SEQ ID NO: 29 - DNA, 44 bp, Artificial Sequence
  primer
ctcatagctaggcgcctgccagggctgcacgtgggtctgttgtg

SEQ ID NO: 30 - DNA, 21 bp, Artificial Sequence
  primer
ggaaacgcaggccacgaaacc

SEQ ID NO: 31 - DNA, 50 bp, Artificial Sequence
  primer
gcttcgcgtctcaggcctgtccagggggcattacagttttgcgtcatgac

SEQ ID NO: 32 - DNA, 21 bp, Artificial Sequence
  primer
caagtctgagcacttgcaccg

SEQ ID NO: 33 - DNA, 47 bp, Artificial Sequence
  primer
ctgttagctctgcgagctccaggggagcgacacttgttggtgttgac

SEQ ID NO: 34 - DNA, 23 bp, Artificial Sequence
  primer
tgatgaaatgaagccacccgtgc

SEQ ID NO: 35 - DNA, 41 bp, Artificial Sequence
  SCO
tcggagccagcgcggcgtaaacccactccagccggctgaca

SEQ ID NO: 36 - DNA, 44 bp, Artificial Sequence
  SCO
tacaacagcagtacggagacgactcatcgccacgagccggttaa

SEQ ID NO: 37 - DNA, 44 bp, Artificial Sequence
  SCO
atttattcttactcgatgttaaatactcacgctaatggagcgca

SEQ ID NO: 38 - DNA, 43 bp, Artificial Sequence
  SCO
tatatatatatattattataaatgctacccagccggctacaag

SEQ ID NO: 39 - DNA, 44 bp, Artificial Sequence
  SCO
aagaataactactacaatctactttgccgcgtgattcgatccca

SEQ ID NO: 40 - DNA, 42 bp, Artificial Sequence
  SCO
ttattattattattattatatattctcatagctgggccgctg

SEQ ID NO: 41 - DNA, 42 bp, Artificial Sequence
  SCO
aatcttcaatgcttaccgtatcagatcgttggcactctgcga

SEQ ID NO: 42 - DNA, 42 bp, Artificial Sequence
  SCO
aaaataaataatataatatatgctcgtatgccgctccatata

SEQ ID NO: 43 - DNA, 43 bp, Artificial Sequence
  SCO
tcggagccagcgcggcgtaacgtacgtgccgtgcatcgttgca

SEQ ID NO: 44 - DNA, 43 bp, Artificial Sequence
  SCO
aagaataactactacaatctactttcgcagtcccgtcgaggaa

SEQ ID NO: 45 - DNA, 41 bp, Artificial Sequence
  SCO
tcggagccagcgcggcgtaatctctcatagctaggcgcctg

SEQ ID NO: 46 - DNA, 41 bp, Artificial Sequence
  SCO
aaaataaataatataatatagtcttcgcgtctcaggcctgt

SEQ ID NO: 47 - DNA, 40 bp, Artificial Sequence
  SCO
aaaataaataatataatatattctgttagctctgcgagct

SEQ ID NO: 48 - DNA, 95 bp, Artificial Sequence
  product
ccactccagccggctgacaccaggacttggtgtgacgctatcagcatgcgtatgggttactatggtgactttgttttcgaccgtgttttgaaaac

SEQ ID NO: 49 - DNA, 122 bp, Artificial Sequence
  product
cgcccaccgcatcccgcgcccctccctcagcaccaggttgaaacaccgcccggaacccgatataatccgcccttcaacatcagtgaaaatctttttttaaccggtcaaaccgaataaggagc

SEQ ID NO: 50 - DNA, 135 bp, Artificial Sequence
  product
actcacgctaatggagcgcaccaggtttagctcctattgccaacgtattggaaaaaaactttggtattgaaaaaggatttatgacaacagtccactcatatacagcagaccaaagattacaagatgctccacaca

SEQ ID NO: 51 - DNA, 251 bp, Artificial Sequence
  product
gctacccagccggctacaagccaggctttatggtgcttatattggtggcatgcaccatgatcgtccttttaaaaagtctgcgaggattgttggtgatgtaatgagtaaattccaccctcatggtgatatggcaatatatgacaccatgtcaagaatggctcaagacttttcattaagataccttttaattgatggtcatggtaattttggttctatagatggtgatagacctgctgcacaacgttatacag

SEQ ID NO: 52 - DNA, 111 bp, Artificial Sequence
  product
tgccgcgtgattcgatcccaccaggtatgtccggcacaacatgcgcttatgtccggcacaacatgcgctctccgcttcccaggtcagctcaactccgaccttcgtaagctc

SEQ ID NO: 53 - DNA, 225 bp, Artificial Sequence
  product
tctcatagctgggccgctgccaggaagtagcatatgatgaagcacacaacaaaatggcgcatactgtgtatttcactaatttctatcgttcatcaaaaccactatttttagatgaagaagacccaattaatccctgttttcaaactattagtatgggtgggggttatgtatctggtgaagtgtatcgttctgattttgaagttgaagcaaatgcacgttgcatta

SEQ ID NO: 54 - DNA, 236 bp, Artificial Sequence
  product
cagatcgttggcactctgcgaccaggttaaagtagcatatgatcaagctcattcaaaaatggcacatactgtctattttacgaatttttatcgttcatctaaacctttatttttagatgaagaagatccaatcaacccctgttttcaaacaattagtatgggtggtggatatgtttcaggtgaaatttatcgttctgattttgaaattaatgatgatgctcgttgtatcattacaa

SEQ ID NO: 55 - DNA, 102 bp, Artificial Sequence
  product
gctcgtatgccgctccatataccaggccaaatctggatcttcctctgcatctgcttctggatcatcaagcagcagcaccagctctgggtccagctcaagctc

SEQ ID NO: 56 - DNA, 187 bp, Artificial Sequence
  product
acgtgccgtgcatcgttgcaccaggcaaccggctccattttggtggagtcgcttgatcgttttgtgatcgtttagtgtgatgatttattatgtctagagagttaagcgataggcttttactggtgtatcactgtaagggcgtattggttggatgccttggtagacaggaccgatgaaggacgtgacg

SEQ ID NO: 57 - DNA, 172 bp, Artificial Sequence
  product
tcgcagtcccgtcgaggaaccaggaggcctggctatccggagaaacagcacacgacttggcgttctgtgtgtcgcgatgtctctgcgcgcagtctggcatctggggcttttgggaagcctcgtgggggctgttcttgccgccacccatcggggacctgcggccaacacaacg

SEQ ID NO: 58 - DNA, 209 bp, Artificial Sequence
  product
ctcatagctaggcgcctgccagggctgcacgtgggtctgttgtgggtagaggtgggcggggagggccccggccccaccgccccccccacaggcggcgcgtgcggagggcggcccgtgcgtccccccggtccccgcgggccgcccgtggcgctcggtgcccccggtatggtattccgcccccaaccccgggtttcgtggcctgcgtttcc

SEQ ID NO: 59 - DNA, 183 bp, Artificial Sequence
  product
gcttcgcgtctcaggcctgtccagggggcattacagttttgcgtcatgacggctttgaagctgacgacctcattgcaaccctagcaaaacgagttgcggctgagcactgtcatgttgtgattatctcctcagataaagatgtacttcagcttgtgtgtgatacggtgcaagtgctcagacttg

SEQ ID NO: 60 - DNA, 183 bp, Artificial Sequence
  product
ctgttagctctgcgagctccaggggagcgacacttgttggtgttgacaagttcggtaacaaatactaccagaagctaggcgatactcaatacggtatgcacagatgggtagagtatgcttcaaaggatcgttacaacgcatctcaagtaccagctgaatggcacgggtggcttcatttcatca

SEQ ID NO: 61 - DNA, 24 bp, Artificial Sequence
  CCTF
cctggtgtcagccggctggagtgg

SEQ ID NO: 62 - DNA, 25 bp, Artificial Sequence
  CCTF
cctggttaaccggctcgtggcgatg

SEQ ID NO: 63 - DNA, 25 bp, Artificial Sequence
  CCTF
cctggtgcgctccattagcgtgagt

SEQ ID NO: 64 - DNA, 25 bp, Artificial Sequence
  CCTF
cctggcttgtagccggctgggtagc

SEQ ID NO: 65 - DNA, 25 bp, Artificial Sequence
  CCTF
cctggtgggatcgaatcacgcggca

SEQ ID NO: 66 - DNA, 24 bp, Artificial Sequence
  CCTF
cctggcagcggcccagctatgaga

SEQ ID NO: 67 - DNA, 26 bp, Artificial Sequence
  CCTF
cctggtcgcagagtgccaacgatctg

SEQ ID NO: 68 - DNA, 26 bp, Artificial Sequence
  CCTF
cctggtatatggagcggcatacgagc

SEQ ID NO: 69 - DNA, 25 bp, Artificial Sequence
  CCTF
cctggtgcaacgatgcacggcacgt

SEQ ID NO: 70 - DNA, 24 bp, Artificial Sequence
  CCTF
cctggttcctcgacgggactgcga

SEQ ID NO: 71 - DNA, 23 bp, Artificial Sequence
  CCTF
cctggcaggcgcctagctatgag

SEQ ID NO: 72 - DNA, 25 bp, Artificial Sequence
  CCTF
cctggacaggcctgagacgcgaagc

SEQ ID NO: 73 - DNA, 23 bp, Artificial Sequence
  CCTF
cctggagctcgcagagctaacag

SEQ ID NO: 74 - DNA, 53 bp, Artificial Sequence
  primer
gcaggagcctctcatctcgccaggctcatttatagacarcttctcactaattc

SEQ ID NO: 75 - DNA, 30 bp, Artificial Sequence
  primer
agttttttctgatccaatytgytctatttc

SEQ ID NO: 76 - DNA, 49 bp, Artificial Sequence
  primer
tcagacggttcgaggctccccaggargatyaagcgtggagtatayatgg

SEQ ID NO: 77 - DNA, 21 bp, Artificial Sequence
  primer
tttgcgtgcytcttcacacgc

SEQ ID NO: 78 - DNA, 46 bp, Artificial Sequence
  primer
aacgcgaatcgaccggatccaggcgcgatgtgtttgccgataaaac

SEQ ID NO: 79 - DNA, 20 bp, Artificial Sequence
  primer
cattgcgtctgccccacttg

SEQ ID NO: 80 - DNA, 51 bp, Artificial Sequence
  primer
aacgcgaatcgaccggatccaggaaacaagaacacctatgcctacatgaac

SEQ ID NO: 81 - DNA, 27 bp, Artificial Sequence
  primer
atgttaacgtccttcctgaagttccac

SEQ ID NO: 82 - DNA, 46 bp, Artificial Sequence
  primer
tagatcggactgcgaatcgccagggagatcgcratctyctgcccga

SEQ ID NO: 83 - DNA, 22 bp, Artificial Sequence
  primer
rgcgtccttagacgccatcatc

SEQ ID NO: 84 - DNA, 49 bp, Artificial Sequence
  primer
atctacagcgtcgcatcacgccaggcgcaatctggctcccarttttgtg

SEQ ID NO: 85 - DNA, 22 bp, Artificial Sequence
  primer
gcgtcaytcgacgccatcytca

SEQ ID NO: 86 - DNA, 51 bp, Artificial Sequence
  primer
cataggtcgaggtcctcacccagggcaaactccggcatctactaatagacg

SEQ ID NO: 87 - DNA, 20 bp, Artificial Sequence
  primer
aagcggtgatccgcacagtg

SEQ ID NO: 88 - DNA, 47 bp, Artificial Sequence
  SCO
tcggccgatcgtccatagagtcaagctcgcaggagcctctcatctcg

SEQ ID NO: 89 - DNA, 45 bp, Artificial Sequence
  SCO
tcacgatgagcgagttgagctacgtatcagacggttcgaggctcc

SEQ ID NO: 90 - DNA, 43 bp, Artificial Sequence
  SCO
tgttcaatatataatgataatatgtaacgcgaatcgaccggat

SEQ ID NO: 91 - DNA, 43 bp, Artificial Sequence; identical to SEQ ID NO: 90
  SCO

SEQ ID NO: 92 - DNA, 42 bp, Artificial Sequence
  SCO
acatttataatacagtattttattagatcggactgcgaatcg

SEQ ID NO: 93 - DNA, 45 bp, Artificial Sequence
  SCO
agctcctgccagtactgccatccatatctacagcgtcgcatcacg

SEQ ID NO: 94 - DNA, 43 bp, Artificial Sequence
  SCO
tagttataatgaataactattattcataggtcgaggtcctcac

SEQ ID NO: 95 - DNA, 105 bp, Artificial Sequence
  product
gcaggagcctctcatctcgccaggctcatttatagacarcttctcactaattcatattcagtagatttacatgatgaaatagarcarattggatcagaaaaaact

SEQ ID NO: 96 - DNA, 114 bp, Artificial Sequence
  product
tcagacggttcgaggctccccaggargatyaagcgtggagtatayatggacctgcttgtctcgggggcaagcccaggcaatgcatggtcccatgcgtgtgaagargcacgcaaa

SEQ ID NO: 97 - DNA, 82 bp, Artificial Sequence
  product
aacgcgaatcgaccggatccaggcgcgatgtgtttgccgataaaacgtaccaaccggagccccaagtggggcagacgcaatg

SEQ ID NO: 98 - DNA, 308 bp, Artificial Sequence
  product
aacgcgaatcgaccggatccaggaaacaagaacacctatgcctacatgaacggtcgggtggcggttcctagcgccctcgatacctacgtaaacatcggggcacggtggtctccagatcccatggacaatgttaaccccttcaatcaccaccgtaacgccggtctgcgctatcgatccatgctcttgggcaacgggcgttacgtacccttccacattcaagtcccccagaagttttttgccattaaaaatctcctcctcttaccgggttcctacacctacgagtggaacttcaggaaggacgttaacat

SEQ ID NO: 99 - DNA, 78 bp, Artificial Sequence
  product
tagatcggactgcgaatcgccagggagatcgcratctyctgcccgaattcgtaaatgatgatggcgtctaaggacgcy

SEQ ID NO: 100 - DNA, 73 bp, Artificial Sequence
  product
atctacagcgtcgcatcacgccaggcgcaatctggctcccarttttgtgaatgargatggcgtcgartgacgc

SEQ ID NO: 101 - DNA, 196 bp, Artificial Sequence
  product
cataggtcgaggtcctcacccagggcaaactccggcatctactaatagacgccggccattcaaacatgaggattacccatgtcgaagacaacaaagaagttcaactctttatgtattgatcttcctcgcgatctttctctcgaaatttaccaatcaattgcttctgtcgctactggaagcggtgatccgcacagtg

SEQ ID NO: 102 - DNA, 24 bp, Artificial Sequence
  CCTF
cctggtgtcagccggctggagtgg

SEQ ID NO: 103 - DNA, 25 bp, Artificial Sequence
  CCTF
cctggttaaccggctcgtggcgatg

SEQ ID NO: 104 - DNA, 25 bp, Artificial Sequence
  CCTF
cctggtgcgctccattagcgtgagt

SEQ ID NO: 105 - DNA, 25 bp, Artificial Sequence
  CCTF
cctggcttgtagccggctgggtagc

SEQ ID NO: 106 - DNA, 25 bp, Artificial Sequence
  CCTF
cctggtgggatcgaatcacgcggca

SEQ ID NO: 107 - DNA, 24 bp, Artificial Sequence
  CCTF
cctggcagcggcccagctatgaga

SEQ ID NO: 108 - DNA, 26 bp, Artificial Sequence
  CCTF
cctggtcgcagagtgccaacgatctg

SEQ ID NO: 109 - DNA, 26 bp, Artificial Sequence
  CCTF
cctggtatatggagcggcatacgagc

SEQ ID NO: 110 - DNA, 25 bp, Artificial Sequence
  CCTF
cctggtgcaacgatgcacggcacgt

SEQ ID NO: 111 - DNA, 24 bp, Artificial Sequence
  CCTF
cctggttcctcgacgggactgcga

SEQ ID NO: 112 - DNA, 23 bp, Artificial Sequence
  CCTF
cctggcaggcgcctagctatgag

SEQ ID NO: 113 - DNA, 25 bp, Artificial Sequence
  CCTF
cctggacaggcctgagacgcgaagc

SEQ ID NO: 114 - DNA, 23 bp, Artificial Sequence
  CCTF
cctggagctcgcagagctaacag

SEQ ID NO: 115 - DNA, 51 bp, Artificial Sequence
  primer
ctctgatagcgactgctcgcaccaggataatataaggggtcggtggaccgg

SEQ ID NO: 116 - DNA, 25 bp, Artificial Sequence
  primer
ctccatgcatgattacagctgggtt

SEQ ID NO: 117 - DNA, 49 bp, Artificial Sequence
  primer
atcggtctcctgaaagctgcgccaggcagaaggtacagacggggagggc

SEQ ID NO: 118 - DNA, 22 bp, Artificial Sequence
  primer
cacctccagccgctcccctaat

SEQ ID NO: 119 - DNA, 51 bp, Artificial Sequence
  primer
ctggcgtagagcacttacgctccaggcaacgataaccgaccaccacaagca

SEQ ID NO: 120 - DNA, 23 bp, Artificial Sequence
  primer
cggggtctgcacagaacagcttt

SEQ ID NO: 121 - DNA, 51 bp, Artificial Sequence
  primer
ctggcgtagagcacttacgctccaggaggacccagctgaacgaccttacaa

SEQ ID NO: 122 - DNA, 25 bp, Artificial Sequence
  primer
ctgtccaccgtccaccgatgttatg

SEQ ID NO: 123 - DNA, 48 bp, Artificial Sequence
  primer
ctggcgtagagcacttacgctccagggctggcaacgtacacgacaacg

SEQ ID NO: 124 - DNA, 22 bp, Artificial Sequence
  primer
gctgtacaacgcgaagggtgtc

SEQ ID NO: 125 - DNA, 51 bp, Artificial Sequence
  primer
ctggcgtagagcacttacgctccaggtccacctatgcaccgaaacctccaa

SEQ ID NO: 126 - DNA, 25 bp, Artificial Sequence
  primer
tgcagtgacgagtccccgtgtagta

SEQ ID NO: 127 - DNA, 49 bp, Artificial Sequence
  primer
ctggcgtagagcacttacgctccagggactgtacaccgtatgcagcgtg

SEQ ID NO: 128 - DNA, 21 bp, Artificial Sequence
  primer
gcgtatcagcagctcatgtaa

SEQ ID NO: 129 - DNA, 49 bp, Artificial Sequence
  primer
ctggcgtagagcacttacgctccaggacaaactcgacgtcgtctcggaa

SEQ ID NO: 130 - DNA, 25 bp, Artificial Sequence
  primer
caggtcaccacaacaaaggctccgt

SEQ ID NO: 131 - DNA, 49 bp, Artificial Sequence
  primer
atcaggacgcagccggttctccaggccaaggacaggtacggctgtcatc

SEQ ID NO: 132 - DNA, 24 bp, Artificial Sequence
  primer
ggtgcccttgaggttgtccaggtg

SEQ ID NO: 133 - DNA, 45 bp, Artificial Sequence
  SCO
gagacgtttaagtccgcgaccgctctctgatagcgactgctcgca

SEQ ID NO: 134 - DNA, 45 bp, Artificial Sequence
  SCO
caggcgacgtccatatggtgcgctatcggtctcctgaaagctgcg

SEQ ID NO: 135 - DNA, 39 bp, Artificial Sequence
  SCO
cccttaggtaacgtctggctggcgtagagcacttacgct

SEQ ID NO: 136 - DNA, 38 bp, Artificial Sequence
  SCO
aaactttaattattgtatatcaggacgcagccggttct

SEQ ID NO: 137 - DNA, 118 bp, Artificial Sequence
  product
ctctgatagcgactgctcgcaccaggataatataaggggtcggtggaccggtcgatgtatgtcttgttgcagatcatcaagaacacgtagagaaacccagctgtaatcatgcatggag

SEQ ID NO: 138 - DNA, 236 bp, Artificial Sequence
  product
atcggtctcctgaaagctgcgccaggcacgacaggaacgactccaacgacgcagagaaacacaagtataatattaagtatgcatggacctaaggcaacattgcaagacattgtattgcatttagagccccaaaatgaaattccggttgaccttctatgtcacgagcaattaagcgactcagaggaagaaaacgatgaaatagatggagttaatcatcaacatttaccagcccgacg

SEQ ID NO: 139 - DNA, 352 bp, Artificial Sequence
  product
ctggcgtagagcacttacgctccaggacgccatgagaggacacaagccaacgttaaaggaatatgttttagatttatatcctgaaccaactgacctatactgctatgagcaattaagtgacagctcagatgaggatgaaggcttggaccggccagatggacaagcacaaccagccacagctgattactacattgtaacctgttgtcacacttgtaacaccacagttcgtttatgtgtcaacagtacagcaagtgacctacgaaccatacagcaactacttatgggcacagtgaatattgtgtgccctacctgtgcacaacaataaacatcatctacaatggccgatcctgaa

SEQ ID NO: 140 - DNA, 419 bp, Artificial Sequence
  product
ctggcgtagagcacttacgctccaggaggacccagctgaacgaccttacaaactgcatgatttgtgcaacgaggtagaagaaagcatccatgaaatttgtttgaattgtgtatactgcaaacaagaattacagcggagtgaggtatatgactttgcatgctatgatttgtgtatagtatatagagaaggccagccatatggagtatgcatgaaatgtttaaaattttattcaaaaataagtgaatatagatggtatagatatagtgtgtatggagaaacgttagaaaaacaatgcaacaaacagttatgtcatttattaattaggtgtattacatgtcaaaaaccgctgtgtccagttgaaaagcaaagacatttagaagaaaaaaaacgattccataacatcggtggacggtggacag

SEQ ID NO: 141 - DNA, 327 bp, Artificial Sequence
  product
ctggcgtagagcacttacgctccagggctggcaacgtacacgacaacgtaacgaaacccaagtgtaataaagccatgcgtggtaatgtaccacaattaaaagatgtagtattgcatttaacaccacagactgaaattgacttgcaatgctacgagcaatttgacagctcagaggaggaggatgaagtagataatatgcgtgaccagctaccagaaagacgggctggacaggctacgtgttacagaattgaagctccgtgttgcaggtgttcaagtgtagtacaactggcagtggaaagcagtggagacacccttcgcgttgtacagc

SEQ ID NO: 142 - DNA, 211 bp, Artificial Sequence
  product
ctggcgtagagcacttacgctccaggtccacctatgcaccgaaacctccaagacctccgcattgtccgtgggtgccaaagacacacacctacaaccaccacagaaacgacgacgaccagacgtcacagactccagaaacaccaagtaccccaacaaccttttgcggggacaacaatccgtggacagtactacacggggactcgtcactgca

SEQ ID NO: 143 - DNA, 167 bp, Artificial Sequence
  product
ctggcgtagagcacttacgctccagggttaagaccgaaaacggtgcatataaaggtagttagaaagaaaagggcaacggcatggcacgctttgaggatcctacacaacgaccatacaaactgcctgacttgagcacaacattgaatattcctctgcatgatattcgc

SEQ ID NO: 144 - DNA, 179 bp, Artificial Sequence
  product
ctggcgtagagcacttacgctccaggatggcgctatttcacaaccctgaggaacggccatacaaattgccagacctgtgcaggacattggacactacattgcatgacgttacaatagagtgtgtctattgcagaaggcaactacaacggacagaggtatatgaatttgcctttagtgac

SEQ ID NO: 145 - DNA, 277 bp, Artificial Sequence
  product
gctcatatgcggcgccatttaccagggcaggttgctatcaaggttacaagacaggtttaaggagaccaatagaaactgggcatgtggagacagagaagactcttgggtttctgataggcactgactctctctgcctattggtctattttcccacccttaggctgctggtggtctacccttggacccagaggttctttgagtcctttggggatctgtccactcctgatgctgttatgggcaaccctaaggtgaaggctcatggcaagaaagtgctcgg

SEQ ID NO: 146 - DNA, 21 bp, Artificial Sequence
  CCTF
tgcgagcagtcgctatcagag

SEQ ID NO: 147 - DNA, 21 bp, Artificial Sequence
  CCTF
cgcagctttcaggagaccgat

SEQ ID NO: 148 - DNA, 21 bp, Artificial Sequence
  CCTF
agcgtaagtgctctacgccag

SEQ ID NO: 149 - DNA, 20 bp, Artificial Sequence
  CCTF
agaaccggctgcgtcctgat

SEQ ID NO: 150 - DNA, 26 bp, Artificial Sequence
  primer
ttgctatggctgacggggaagaatgg

SEQ ID NO: 151 - DNA, 56 bp, Artificial Sequence
  primer
gccccgttgagagcacgaatccaggggggtgaatcttctgcttaatgtgaagacac

SEQ ID NO: 152 - DNA, 26 bp, Artificial Sequence
  primer
gggcaccatgcagtaccaaacggaac

SEQ ID NO: 153 - DNA, 52 bp, Artificial Sequence
  primer
ccgtggcgcgaacttatcgaccaggatcacactgagggtctcccaatagagc

SEQ ID NO: 154 - DNA, 29 bp, Artificial Sequence
  primer
tcaaagactaagtggtgccatggatgaac

SEQ ID NO: 155 - DNA, 50 bp, Artificial Sequence
  primer
aagtgacctgccattgcgcgccaggtatgtctacagcagagggacccagc

SEQ ID NO: 156 - DNA, 49 bp, Artificial Sequence
  primer
ggcttagagcaccgcgtcattccaggtgtcgctactggaagcggtgatc

SEQ ID NO: 157 - DNA, 24 bp, Artificial Sequence
  primer
gcgatagctaaggtacgacgggtc

SEQ ID NO: 158 - DNA, 29 bp, Artificial Sequence
  primer
gtagattcgatccatgctcctctactacc

SEQ ID NO: 159 - DNA, 55 bp, Artificial Sequence
  primer
cgtcttacatgcgcaagcggccaggtgatattgagttcggtaatgcaagatctgc

SEQ ID NO: 160 - DNA, 27 bp, Artificial Sequence
  primer
ccatagagatggcaatagatgaagagc

SEQ ID NO: 161 - DNA, 52 bp, Artificial Sequence
  primer
aggcgttccgcttcaacgagccaggttgtcagattctgtagcttgctcagtc

SEQ ID NO: 162 - DNA, 29 bp, Artificial Sequence
  primer
ggtggtgatcccaacttgttatatcgaag

SEQ ID NO: 163 - DNA, 56 bp, Artificial Sequence
  primer
tccgtctgcgaagatctgagcccaggttcaatctatcrtctgacagatcttgaagt

SEQ ID NO: 164 - DNA, 54 bp, Artificial Sequence
  primer
gtgtcacgacgcgcgaatctccaggagatcgtgaccagtataatagctcaacac

SEQ ID NO: 165 - DNA, 28 bp, Artificial Sequence
  primer
tttcagacaatgcagggataacaccagc

SEQ ID NO: 166 - DNA, 50 bp, Artificial Sequence
  primer
cccagaacgatttgcggcgtccaggcttggtcctctcttaggaggcaagc

SEQ ID NO: 167 - DNA, 22 bp, Artificial Sequence
  primer
aggatgcttcggagtacctgag

SEQ ID NO: 168 - DNA, 45 bp, Artificial Sequence
  primer
tgcattgccgtcgcagagacccaggcaacgggcacgaagcgcatc

SEQ ID NO: 169 - DNA, 28 bp, Artificial Sequence
  primer
gccctaatgataagacaggcagttgtgg

SEQ ID NO: 170 - DNA, 52 bp, Artificial Sequence
  primer
atgcgcttggattgccgatgccaggagccctgttagttctggatgctgaaca

SEQ ID NO: 171 - DNA, 35 bp, Artificial Sequence
  SCO
cttatagattatattgccccgttgagagcacgaat

SEQ ID NO: 172 - DNA, 42 bp, Artificial Sequence
  SCO
ctaagtaagcctatatcgaattccgtggcgcgaacttatcga

SEQ ID NO: 173 - DNA, 42 bp, Artificial Sequence
  SCO
cgtactgcactcgcctacgactaagtgacctgccattgcgcg

SEQ ID NO: 174 - DNA, 35 bp, Artificial Sequence
  SCO
cttataagttacatggcttagagcaccgcgtcatt

SEQ ID NO: 175 - DNA, 34 bp, Artificial Sequence
  SCO
ctaattgtaatactcgtcttacatgcgcaagcgg

SEQ ID NO: 176 - DNA, 42 bp, Artificial Sequence
  SCO
ctaatcgtatgagatctatgataggcgttccgcttcaacgag

SEQ ID NO: 177 - DNA, 35 bp, Artificial Sequence
  SCO
tcatagacatttattccgtctgcgaagatctgagc

SEQ ID NO: 178 - DNA, 42 bp, Artificial Sequence
  SCO
tacgaatctgacctagtaagatgtgtcacgacgcgcgaatct

SEQ ID NO: 179 - DNA, 42 bp, Artificial Sequence
  SCO
tgccactaacaggccgctagatcccagaacgatttgcggcgt

SEQ ID NO: 180 - DNA, 41 bp, Artificial Sequence
  SCO
tcgagcgtgcgccagatccattgcattgccgtcgcagagac

SEQ ID NO: 181 - DNA, 42 bp, Artificial Sequence
  SCO
tcgactgtgcctgcgtccgtatatgcgcttggattgccgatg

SEQ ID NO: 182 - DNA, 219 bp, Artificial Sequence
  product
ttgctatggctgacggggaagaatggtttgtacccaaacctgagcatgtcctatgtaaacaacaaagagaaagaagtccttgtgctatggggtgttcatcacccacctaacatagggaaccaaagggccctctaccatacagaaaatgcttatgtctctgtagtgtcttcacattatagcagaagattcacccccctggattcgtgctctcaacggggc

SEQ ID NO: 183 - DNA, 211 bp, Artificial Sequence
  product
gggcaccatgcagtaccaaacggaacgatagtgaaaacaatcacaaatgaccaaattgaagttactaatgctactgagttggttcagaattcctcaataggtgaaatatgcgacagtcctcatcagatccttgatggagagaactgcacactaatagatgctctattgggagaccctcagtgtgatcctggtcgataagttcgcgccacgg

SEQ ID NO: 184 - DNA, 236 bp, Artificial Sequence
  product
tcaaagactaagtggtgccatggatgaactccacaacgaaatactcgagctggatgaaaaagtggatgacctcagagctgacactataagctcacaaatagaacttgcagtcttgctttccaacgaaggaataataaacagtgaagatgagcatctattggcacttgagagaaaactaaagaaaatgctgggtccctctgctgtagacatacctggcgcgcaatggcaggtcactt

SEQ ID NO: 185 - DNA, 161 bp, Artificial Sequence
  product
ggcttagagcaccgcgtcattccaggtgtcgctactggaagcggtgatccgcacagtgacgactttacagcaattgcttacttaagggacgaattgctcgcaaagcatccgaccttaggttctggtaatgacgaggcgacccgtcgtaccttagctatcgc

SEQ ID NO: 186 - DNA, 244 bp, Artificial Sequence
  product
gtagattcgatccatgctcctctactaccatggtccagccgactgagacaagggatgatatataatgccaataaagtagctctggcaccccaatgtctcccagtcgacaaagatatcagattcagagttgtatttgtcaacggaacatcactgggtacaatcacaattgccaaggtcccaaaaactcttgcagatcttgcattaccgaactcaatatcacctggccgcttgcgcatgtaagacg

SEQ ID NO: 187 - DNA, 179 bp, Artificial Sequence
  product
ccatagagatggcaatagatgaagagccagaacaattcgaacatagagcagaccaagaacaagatggggaacctcaatcatctataatccaatatgcttgggcagaaggaaacagaagcgatgaccggactgagcaagctacagaatctgacaacctggctcgttgaagcggaacgcct

SEQ ID NO: 188 - DNA, 178 bp, Artificial Sequence
  product
ggtggtgatcccaacttgttatatcgaagtttctatagaagaactcctgatttcctcacagaggctatagttcactctgtgttcatacttagttattatacaaaccatgatttaaaggataaacttcaagatctgtcagaygatagattgaacctgggctcagatcttcgcagacgga

SEQ ID NO: 189 - DNA, 138 bp, Artificial Sequence
  product
ggtggtgatcctaatttgttatatcgaagcttttataggagaactccagacttccttacagaagctatagtacattcagtgttcgtgttgagctattatactggtcacgatctcctggagattcgcgcgtcgtgacac

SEQ ID NO: 190 - DNA, 328 bp, Artificial Sequence
  product
tttcagacaatgcagggataacaccagcaatatcattggacctaatgactgatgctgaactggccagagctgtatcatacatgccaacatctgcagggcagataaagctgatgttggagaaccgcgcaatggtaaggagaaaaggatttggaatcctaataggggtctacggaagctctgtgatttacatggttcaattgccgatctttggtgtcatagatacaccttgttggataatcaaggcagctccctcttgctcagaaaaaaacgggaattatgcttgcctcctaagagaggaccaagcctggacgccgcaaatcgttctggg

SEQ ID NO: 191 - DNA, 187 bp, Artificial Sequence
  product
aggatgcttcggagtacctgagtccgggtctggtgcagttcgcccgtgcaacagacacctacttcagtatggggaacaagtttagaaaccccacagtggcgcccacccacgatgtgaccaccgaccgtagccagcgactgatgctgcgcttcgtgcccgttgcctgggtctctgcgacggcaatgca

SEQ ID NO: 192 - DNA, 290 bp, Artificial Sequence
  product
gccctaatgataagacaggcagttgtggtccagtatcgtctaatggagcaaatggagtaaaaggattttcattcaaatacggcaatggtgtttggatagggagaactaaaagcattagttcaagaaaaggttttgagatgatttgggatccgaatggatggactgggactgacaataaattctcaataaagcaagatatcgtaggaataaatgagtggtcagggtatagcgggagttttgttcagcatccagaactaacagggctcctggcatcggcaatccaagcgcat

SEQ ID NO: 193 - DNA, 20 bp, Artificial Sequence
  CCTF
attcgtgctctcaacggggc

SEQ ID NO: 194 - DNA, 20 bp, Artificial Sequence
  CCTF
tcgataagttcgcgccacgg

SEQ ID NO: 195 - DNA, 20 bp, Artificial Sequence
  CCTF
cgcgcaatggcaggtcactt

SEQ ID NO: 196 - DNA, 21 bp, Artificial Sequence
  CCTF
aatgacgcggtgctctaagcc

SEQ ID NO: 197 - DNA, 20 bp, Artificial Sequence
  CCTF
ccgcttgcgcatgtaagacg

SEQ ID NO: 198 - DNA, 20 bp, Artificial Sequence
  CCTF
ctcgttgaagcggaacgcct

SEQ ID NO: 199 - DNA, 21 bp, Artificial Sequence
  CCTF
gctcagatcttcgcagacgga

SEQ ID NO: 200 - DNA, 20 bp, Artificial Sequence
  CCTF
agattcgcgcgtcgtgacac

SEQ ID NO: 201 - DNA, 20 bp, Artificial Sequence
  CCTF
acgccgcaaatcgttctggg

SEQ ID NO: 202 - DNA, 20 bp, Artificial Sequence
  CCTF
gtctctgcgacggcaatgca

SEQ ID NO: 203 - DNA, 20 bp, Artificial Sequence
  CCTF
catcggcaatccaagcgcat

SEQ ID NO: 204 - DNA, 57 bp, Artificial Sequence
  primer
acgaggcctgtccgcttactagccaggctggtcctcatccaacagctcttctatcgc

SEQ ID NO: 205 - DNA, 59 bp, Artificial Sequence
  primer
ccgggtacgctaagtccgctatccaggttctggtcctcatccaacagctcttctatcgt

SEQ ID NO: 206 - DNA, 27 bp, Artificial Sequence
  primer
gacccatgggactctggagagcgtgaa

SEQ ID NO: 207 - DNA, 54 bp, Artificial Sequence
  primer
gctcatatgcggcgccatttaccagggcaggttgctatcaaggttacaagacag

SEQ ID NO: 208 - DNA, 24 bp, Artificial Sequence
  primer
ccgagcactttcttgccatgagcc

SEQ ID NO: 209 - DNA, 44 bp, Artificial Sequence
  SCO
gtagcacgcttcgaatggctatacgaggcctgtccgcttactag

SEQ ID NO: 210 - DNA, 45 bp, Artificial Sequence
  SCO
gatacggaggtccgaaggcagtgttggttaccctaacgcgccgga

SEQ ID NO: 211 - DNA, 45 bp, Artificial Sequence
  SCO
attagtttaactattatattttatgctcatatgcggcgccattta

SEQ ID NO: 212 - DNA, 139 bp, Artificial Sequence
  product
acgaggcctgtccgcttactagccaggctggtcctcatccaacagctcttctatcacgtgttcgaaagtgtcagccaatgatgtcaagcctcttgaacctgccttgggcccattcacgctctccagagtcccatgggtc

SEQ ID NO: 213 - DNA, 141 bp, Artificial Sequence
  product
ccgggtacgctaagtccgctatccaggttctggtcctcatccaacagctcttctatcacgtgttcgaaagtgtcagccaatgatgtcaagcctcttgaacctgccttgggcccattcacgctctccagagtcccatgggtc

SEQ ID NO: 214 - DNA, 277 bp, Artificial Sequence; identical to SEQ ID NO: 145
  product

SEQ ID NO: 215 - DNA, 22 bp, Artificial Sequence
  CCTF
ctagtaagcggacaggcctcgt

SEQ ID NO: 216 - DNA, 22 bp, Artificial Sequence
  CCTF
atagcggacttagcgtacccgg

SEQ ID NO: 217 - DNA, 20 bp, Artificial Sequence
  CCTF
taaatggcgccgcatatgag

SEQ ID NO: 218 - DNA, 48 bp, Artificial Sequence
  primer
ctcatcgccacgagccggttaaccaggttgaaacaccgcccggaaccc

SEQ ID NO: 219 - DNA, 23 bp, Artificial Sequence
  primer
gctccttattcggtttgaccggt

SEQ ID NO: 220 - DNA, 55 bp, Artificial Sequence
  primer
gctcgcaggtacggcaccattcaccaggcagaaggtatgataacaacggtagagc

SEQ ID NO: 221 - DNA, 21 bp, Artificial Sequence
  primer
cccctttgcaccgttgagggg

SEQ ID NO: 222 - DNA, 57 bp, Artificial Sequence
  primer
agtcgattatgtctgaggccgcgccaggttaaagtagcatatgatcaagctcattca

SEQ ID NO: 223 - DNA, 35 bp, Artificial Sequence
  primer
gatcctgacatataatcattatctccttttataaa

SEQ ID NO: 224 - DNA, 23 bp, Artificial Sequence
  SCO
tctcatcgccacgagccggttaa

SEQ ID NO: 225 - DNA, 23 bp, Artificial Sequence
  SCO
tgtcgcaggtacggcaccattca

SEQ ID NO: 226 - DNA, 24 bp, Artificial Sequence
  SCO
tagtcgattatgtctgaggccgcg

SEQ ID NO: 227 - DNA, 112 bp, Artificial Sequence
  product
ctcatcgccacgagccggttaaccaggttgaaacaccgcccggaacccgatataatccgcccttcaacatcagtgaaaatctttttttaaccggtcaaaccgaataaggagc

SEQ ID NO: 228 - DNA, 109 bp, Artificial Sequence
  product
gctcgcaggtacggcaccattcaccaggcagaaggtatgataacaacggtagagctttatatgatattaacttagcaaaaatggaaaacccctcaacggtgcaaagggg

SEQ ID NO: 229 - DNA, 115 bp, Artificial Sequence
  product
agtcgattatgtctgaggccgcgccagggtttctgtacacgatccaattyacaaataacatttacaattcgtaaaatttttttataaaaggagataatgattatatgtcaggatc

SEQ ID NO: 230 - DNA, 27 bp, Artificial Sequence
  CCTF
cctggttaaccggctcgtggcgatgag

SEQ ID NO: 231 - DNA, 28 bp, Artificial Sequence
  CCTF
cctggtgaatggtgccgtacctgcgagc

SEQ ID NO: 232 - DNA, 28 bp, Artificial Sequence
  CCTF
cctggcgcggcctcagacataatcgact